European Patent Specification EP 3 159 352 B1, published August 2, 2023. Title: STITCHED POLYPEPTIDES. Applicant: Verdine, Gregory L Kim, Young-Woo. The sequence listing filed with the application follows.

SEQUENCE LISTING (128 sequences)

SEQ ID NO: 1 - protein, 15 aa, Artificial Sequence
  synthetic peptide synthesized by Fmoc-based solid phase peptide synthesis
EWAETAAAKFLAAHA

SEQ ID NO: 2 - protein, 15 aa, Artificial Sequence
  synthetic peptide synthesized by Fmoc-based solid phase peptide synthesis
  MISC_FEATURE (8)..(8): Xaa represents 2-amino-2-(pent-4-enyl)hept-6-enoic acid or a stapled derivative
EWAETAAXKFLAAHA

SEQ ID NO: 3 - protein, 15 aa, Artificial Sequence
  synthetic peptide synthesized by Fmoc-based solid phase peptide synthesis
  misc_feature (4)..(4): Xaa represents (S)-2-amino-2-methylhept-6-enoic acid or a stapled derivative
  misc_feature (15)..(15): Xaa represents (S)-2-amino-2-methyldec-9-enoic acid or a stapled derivative
EWAXTAAAKFLAAHX

SEQ ID NO: 4 - protein, 15 aa, Artificial Sequence
  synthetic peptide synthesized by Fmoc-based solid phase peptide synthesis
  misc_feature (4)..(4): Xaa represents (S)-2-amino-2-methylhept-6-enoic acid or a stapled derivative
  misc_feature (8)..(8): Xaa represents (R)-2-amino-2-methylhept-6-enoic acid or a stapled derivative
EWAXTAAXKFLAAHA

SEQ ID NO: 5 - protein, 15 aa, Artificial Sequence
  synthetic peptide synthesized by Fmoc-based solid phase peptide synthesis
  misc_feature (8)..(8): Xaa represents (S)-2-amino-2-methylhept-6-enoic acid or a stapled derivative
  misc_feature (15)..(15): Xaa represents (S)-2-amino-2-methyldec-9-enoic acid or a stapled derivative
EWAETAAXKFLAAHX

SEQ ID NO: 6 - protein, 15 aa, Artificial Sequence
  synthetic peptide synthesized by Fmoc-based solid phase peptide synthesis
  misc_feature (4)..(4): Xaa represents (S)-2-amino-2-methylhept-6-enoic acid or a stapled derivative
  misc_feature (8)..(8): Xaa represents (S)-2-amino-2-methylhept-6-enoic acid or a stapled derivative
EWAXTAAXKFLAAHA

SEQ ID NO: 7 - protein, 15 aa, Artificial Sequence
  synthetic peptide synthesized by Fmoc-based solid phase peptide synthesis
  misc_feature (8)..(8): Xaa represents (R)-2-amino-2-methylhept-6-enoic acid or a stapled derivative
  misc_feature (15)..(15): Xaa represents (S)-2-amino-2-methyldec-9-enoic acid or a stapled derivative
EWAETAAXKFLAAHX

SEQ ID NO: 8 - protein, 15 aa, Artificial Sequence
  synthetic peptide synthesized by Fmoc-based solid phase peptide synthesis
  misc_feature (4)..(4): Xaa represents (S)-2-amino-2-methylhept-6-enoic acid or a stapled derivative
  misc_feature (8)..(8): Xaa represents (S)-2-amino-2-methylhept-6-enoic acid or a stapled derivative
  misc_feature (15)..(15): Xaa represents alpha-methyl-Alanine
EWAXTAAXKFLAAHX

SEQ ID NO: 9 - protein, 15 aa, Artificial Sequence
  synthetic peptide synthesized by Fmoc-based solid phase peptide synthesis
  misc_feature (4)..(4): Xaa represents alpha-methyl-Alanine
  misc_feature (8)..(8): Xaa represents (R)-2-amino-2-methylhept-6-enoic acid or a stapled derivative
  misc_feature (15)..(15): Xaa represents (S)-2-amino-2-methyldec-9-enoic acid or a stapled derivative
EWAXTAAXKFLAAHX

SEQ ID NO: 10 - protein, 15 aa, Artificial Sequence
  synthetic peptide synthesized by Fmoc-based solid phase peptide synthesis
  misc_feature (4)..(4): Xaa represents (S)-2-amino-2-methylhept-6-enoic acid or a stapled derivative
  misc_feature (8)..(8): Xaa represents 2-amino-2-(pent-4-enyl)hept-6-enoic acid or a stapled derivative
  misc_feature (15)..(15): Xaa represents (S)-2-amino-2-methyldec-9-enoic acid or a stapled derivative
EWAXTAAXKFLAAHX

SEQ ID NO: 11 - protein, 15 aa, Artificial Sequence
  synthetic peptide synthesized by Fmoc-based solid phase peptide synthesis
  misc_feature (4)..(4): Xaa represents (S)-2-amino-2-methylhept-6-enoic acid or a stapled derivative
  misc_feature (8)..(8): Xaa represents 2-amino-2-(pent-4-enyl)hept-6-enoic acid or a stapled derivative
  misc_feature (12)..(12): Xaa represents (R)-2-amino-2-methylhept-6-enoic acid or a stapled derivative
EWAXTAAXKFLXAHA

SEQ ID NO: 12 - protein, 15 aa, Artificial Sequence
  synthetic peptide synthesized by Fmoc-based solid phase peptide synthesis
  misc_feature (1)..(1): Xaa represents (R)-2-amino-2-methyldec-9-enoic acid or a stapled derivative
  misc_feature (8)..(8): Xaa represents 2-amino-2-(pent-4-enyl)hept-6-enoic acid or a stapled derivative
  misc_feature (12)..(12): Xaa represents (R)-2-amino-2-methylhept-6-enoic acid or a stapled derivative
XWAETAAXKFLXAHA

SEQ ID NO: 13 - protein, 15 aa, Artificial Sequence
  synthetic peptide synthesized by Fmoc-based solid phase peptide synthesis
  misc_feature (1)..(1): Xaa represents (R)-2-amino-2-methyldec-9-enoic acid or a stapled derivative
  misc_feature (8)..(8): Xaa represents 2-amino-2-(pent-4-enyl)hept-6-enoic acid or a stapled derivative
  misc_feature (15)..(15): Xaa represents (S)-2-amino-2-methyldec-9-enoic acid or a stapled derivative
XWAETAAXKFLAAHX

SEQ ID NO: 14 - protein, 15 aa, Artificial Sequence
  synthetic peptide synthesized by Fmoc-based solid phase peptide synthesis
  misc_feature (4)..(4): Xaa represents (R)-2-amino-2-methylhept-6-enoic acid or a stapled derivative
  misc_feature (8)..(8): Xaa represents 2-amino-2-(pent-4-enyl)hept-6-enoic acid or a stapled derivative
  misc_feature (12)..(12): Xaa represents (S)-2-amino-2-methylhept-6-enoic acid or a stapled derivative
EWAXTAAXKFLXAHA

SEQ ID NO: 15 - protein, 16 aa, Artificial Sequence
  synthetic peptide synthesized by Fmoc-based solid phase peptide synthesis
  misc_feature (1)..(1): Xaa represents (S)-2-amino-2-methylhept-6-enoic acid or a stapled derivative
  misc_feature (5)..(5): Xaa represents 2-amino-2-(pent-4-enyl)hept-6-enoic acid or a stapled derivative
  misc_feature (9)..(9): Xaa represents 2-amino-2-(pent-4-enyl)hept-6-enoic acid or a stapled derivative
  misc_feature (13)..(13): Xaa represents (S)-2-amino-2-methylhept-6-enoic acid or a stapled derivative
XEWAXTAAXKFLXAHA

SEQ ID NO: 16 - protein, 15 aa, Artificial Sequence
  synthetic peptide synthesized by Fmoc-based solid phase peptide synthesis -linker1
  misc_feature (4)..(4): Xaa represents (S)-2-amino-2-methylhept-6-enoic acid or a stapled derivative
  misc_feature (8)..(8): Xaa represents 2-amino-2-(pent-4-enyl)hept-6-enoic acid or a stapled derivative
  misc_feature (15)..(15): Xaa represents (S)-2-amino-2-methyldec-9-enoic acid or a stapled derivative
EWAXTAAXKFLAAHX

SEQ ID NO: 17 - protein, 15 aa, Artificial Sequence
  synthetic peptide synthesized by Fmoc-based solid phase peptide synthesis -linker1
  misc_feature (1)..(1): Xaa represents (R)-2-amino-2-methyldec-9-enoic acid or a stapled derivative
  misc_feature (8)..(8): Xaa represents 2-amino-2-(pent-4-enyl)hept-6-enoic acid or a stapled derivative
  misc_feature (15)..(15): Xaa represents (S)-2-amino-2-methyldec-9-enoic acid or a stapled derivative
XWAETAAXKFLAAHX

SEQ ID NO: 18 - protein, 15 aa, Artificial Sequence
  synthetic peptide synthesized by Fmoc-based solid phase peptide synthesis -linker1
  misc_feature (4)..(4): Xaa represents (S)-2-amino-2-methylhept-6-enoic acid or a stapled derivative
  misc_feature (8)..(8): Xaa represents 2-amino-2-(pent-4-enyl)hept-6-enoic acid or a stapled derivative
  misc_feature (12)..(12): Xaa represents (R)-2-amino-2-methylhept-6-enoic acid or a stapled derivative
EWAXTAAXKFLXAHA

SEQ ID NO: 19 - protein, 15 aa, Artificial Sequence
  synthetic peptide synthesized by Fmoc-based solid phase peptide synthesis
  misc_feature (1)..(1): Xaa represents (R)-2-amino-2-methyldec-9-enoic acid or a stapled derivative
  misc_feature (8)..(8): Xaa represents 2-amino-2-(pent-4-enyl)hept-6-enoic acid or a stapled derivative
  misc_feature (15)..(15): Xaa represents (S)-2-amino-2-methyldec-9-enoic acid or a stapled derivative
XWAETAAXKFLAAHX

SEQ ID NO: 20 - protein, 15 aa, Artificial Sequence
  synthetic peptide synthesized by Fmoc-based solid phase peptide synthesis
  misc_feature (4)..(4): Xaa represents (S)-2-amino-2-methylhept-6-enoic acid or a stapled derivative
  misc_feature (8)..(8): Xaa represents 2-amino-2-(pent-4-enyl)hept-6-enoic acid or a stapled derivative
  misc_feature (12)..(12): Xaa represents (R)-2-amino-2-methylhept-6-enoic acid or a stapled derivative
EWAXTAAXKFLXAHA

SEQ ID NO: 21 - protein, 15 aa, Artificial Sequence
  synthetic peptide synthesized by Fmoc-based solid phase peptide synthesis
EWAETAAAKFLAAHA

SEQ ID NO: 22 - protein, 15 aa, Artificial Sequence
  synthetic peptide synthesized by Fmoc-based solid phase peptide synthesis
  misc_feature (4)..(4): Xaa represents (R)-2-amino-2-methylhept-6-enoic acid or a stapled derivative
  misc_feature (8)..(8): Xaa represents (R)-2-amino-2-methylhept-6-enoic acid or a stapled derivative
  misc_feature (15)..(15): Xaa represents alpha-methyl-Alanine
EWAXTAAXKFLAAHX

SEQ ID NO: 23 - protein, 15 aa, Artificial Sequence
  synthetic peptide synthesized by Fmoc-based solid phase peptide synthesis
  misc_feature (4)..(4): Xaa represents (S)-2-amino-2-methylhept-6-enoic acid or a stapled derivative
  misc_feature (8)..(8): Xaa represents (S)-2-amino-2-methylhept-6-enoic acid or a stapled derivative
  misc_feature (15)..(15): Xaa represents alpha-methyl-Alanine
EWAXTAAXKFLAAHX

SEQ ID NO: 24 - protein, 15 aa, Artificial Sequence
  synthetic peptide synthesized by Fmoc-based solid phase peptide synthesis
  misc_feature (4)..(4): Xaa represents alpha-methyl-Alanine
  misc_feature (8)..(8): Xaa represents (R)-2-amino-2-methylhept-6-enoic acid or a stapled derivative
  misc_feature (15)..(15): Xaa represents (S)-2-amino-2-methyldec-9-enoic acid or a stapled derivative
EWAXTAAXKFLAAHX

SEQ ID NO: 25 - protein, 15 aa, Artificial Sequence
  synthetic peptide synthesized by Fmoc-based solid phase peptide synthesis
  misc_feature (4)..(4): Xaa represents (S)-2-amino-2-methylhept-6-enoic acid or a stapled derivative
  misc_feature (8)..(8): Xaa represents 2-amino-2-(pent-4-enyl)hept-6-enoic acid or a stapled derivative
  misc_feature (15)..(15): Xaa represents (S)-2-amino-2-methyldec-9-enoic acid or a stapled derivative
EWAXTAAXKFLAAHX

SEQ ID NO: 26 - protein, 15 aa, Artificial Sequence
  synthetic peptide synthesized by Fmoc-based solid phase peptide synthesis
  misc_feature (4)..(4): Xaa represents alpha-methyl-Alanine
  misc_feature (8)..(8): Xaa represents alpha-methyl-Alanine
  misc_feature (15)..(15): Xaa represents alpha-methyl-Alanine
EWSXTDNXKQEADRX

SEQ ID NO: 27 - protein, 15 aa, Artificial Sequence
  synthetic peptide synthesized by Fmoc-based solid phase peptide synthesis
  misc_feature (4)..(4): Xaa represents (S)-2-amino-2-methylhept-6-enoic acid or a stapled derivative
  misc_feature (8)..(8): Xaa represents 2-amino-2-(pent-4-enyl)hept-6-enoic acid or a stapled derivative
  misc_feature (15)..(15): Xaa represents (S)-2-amino-2-methyldec-9-enoic acid or a stapled derivative
EWSXTDNXKQEADRX

SEQ ID NO: 28 - protein, 15 aa, Artificial Sequence
  synthetic peptide synthesized by Fmoc-based solid phase peptide synthesis
  misc_feature (4)..(4): Xaa represents (S)-2-amino-2-methylhept-6-enoic acid or a stapled derivative
  misc_feature (8)..(8): Xaa represents 2-amino-2-(pent-4-enyl)hept-6-enoic acid or a stapled derivative
  misc_feature (12)..(12): Xaa represents (R)-2-amino-2-methylhept-6-enoic acid or a stapled derivative
EWSXTDNXKQEXDRA

SEQ ID NO: 29 - protein, 17 aa, Artificial Sequence
  synthetic peptide synthesized by Fmoc-based solid phase peptide synthesis
  misc_feature (4)..(4): Xaa represents (S)-2-amino-2-methylhept-6-enoic acid or a stapled derivative
  misc_feature (8)..(8): Xaa represents 2-amino-2-(pent-4-enyl)hept-6-enoic acid or a stapled derivative
  misc_feature (15)..(15): Xaa represents (S)-2-amino-2-methyldec-9-enoic acid or a stapled derivative
TRQXRRNXRRRWREXQR

SEQ ID NO: 30 - protein, 17 aa, Artificial Sequence
  synthetic peptide synthesized by Fmoc-based solid phase peptide synthesis
  misc_feature (4)..(4): Xaa represents (S)-2-amino-2-methylhept-6-enoic acid or a stapled derivative
  misc_feature (8)..(8): Xaa represents 2-amino-2-(pent-4-enyl)hept-6-enoic acid or a stapled derivative
  misc_feature (12)..(12): Xaa represents (S)-2-amino-2-methylhept-6-enoic acid or a stapled derivative
TRQXRRNXWRRXRERQR

SEQ ID NO: 31 - protein, 17 aa, Artificial Sequence
  synthetic peptide synthesized by Fmoc-based solid phase peptide synthesis
  misc_feature (4)..(4): Xaa represents (S)-2-amino-2-methylhept-6-enoic acid or a stapled derivative
  misc_feature (8)..(8): Xaa represents 2-amino-2-(pent-4-enyl)hept-6-enoic acid or a stapled derivative
  misc_feature (15)..(15): Xaa represents (S)-2-amino-2-methyldec-9-enoic acid or a stapled derivative
TRQXRRNXRRRWREXQR

SEQ ID NO: 32 - protein, 17 aa, Artificial Sequence
  synthetic peptide synthesized by Fmoc-based solid phase peptide synthesis
  misc_feature (4)..(4): Xaa represents (S)-2-amino-2-methylhept-6-enoic acid or a stapled derivative
  misc_feature (8)..(8): Xaa represents 2-amino-2-(pent-4-enyl)hept-6-enoic acid or a stapled derivative
  misc_feature (12)..(12): Xaa represents (R)-2-amino-2-methylhept-6-enoic acid or a stapled derivative
TRQXRRNXWRRXRERQR

SEQ ID NO: 33 - protein, 15 aa, Artificial Sequence
  synthetic peptide synthesized by Fmoc-based solid phase peptide synthesis
  misc_feature (3)..(3): Xaa represents (S)-2-amino-2-methylhept-6-enoic acid or a stapled derivative
  misc_feature (7)..(7): Xaa represents 2-amino-2-(pent-4-enyl)hept-6-enoic acid or a stapled derivative
  misc_feature (14)..(14): Xaa represents (S)-2-amino-2-methyldec-9-enoic acid or a stapled derivative
ILXMAVXHMKSLRXT

SEQ ID NO: 34 - protein, 15 aa, Artificial Sequence
  synthetic peptide synthesized by Fmoc-based solid phase peptide synthesis
  misc_feature (7)..(7): Xaa represents (S)-2-amino-2-methylhept-6-enoic acid or a stapled derivative
  misc_feature (11)..(11): Xaa represents 2-amino-2-(pent-4-enyl)hept-6-enoic acid or a stapled derivative
  misc_feature (15)..(15): Xaa represents (R)-2-amino-2-methylhept-6-enoic acid or a stapled derivative
ILRMAVXHMKXLRGX

SEQ ID NO: 35 - protein, 15 aa, Artificial Sequence
  synthetic peptide synthesized by Fmoc-based solid phase peptide synthesis
  misc_feature (3)..(3): Xaa represents (S)-2-amino-2-methylhept-6-enoic acid or a stapled derivative
  misc_feature (7)..(7): Xaa represents 2-amino-2-(pent-4-enyl)hept-6-enoic acid or a stapled derivative
  misc_feature (14)..(14): Xaa represents (S)-2-amino-2-methyldec-9-enoic acid or a stapled derivative
ILXMAVXHMKSLRXT

SEQ ID NO: 36 - protein, 15 aa, Artificial Sequence
  synthetic peptide synthesized by Fmoc-based solid phase peptide synthesis
  misc_feature (7)..(7): Xaa represents (S)-2-amino-2-methylhept-6-enoic acid or a stapled derivative
  misc_feature (11)..(11): Xaa represents 2-amino-2-(pent-4-enyl)hept-6-enoic acid or a stapled derivative
ILRMAVXHMKXLRGR

SEQ ID NO: 37 - protein, 16 aa, Artificial Sequence
  synthetic peptide synthesized by Fmoc-based solid phase peptide synthesis
  misc_feature (3)..(3): Xaa represents (S)-2-amino-2-methylhept-6-enoic acid or a stapled derivative
  misc_feature (7)..(7): Xaa represents 2-amino-2-(pent-4-enyl)hept-6-enoic acid or a stapled derivative
  misc_feature (14)..(14): Xaa represents (S)-2-amino-2-methyldec-9-enoic acid or a stapled derivative
LSXETFXDLWKLLXEN

SEQ ID NO: 38 - protein, 16 aa, Artificial Sequence
  synthetic peptide synthesized by Fmoc-based solid phase peptide synthesis
  misc_feature (3)..(3): Xaa represents (S)-2-amino-2-methylhept-6-enoic acid or a stapled derivative
  misc_feature (7)..(7): Xaa represents 2-amino-2-(pent-4-enyl)hept-6-enoic acid or a stapled derivative
  misc_feature (14)..(14): Xaa represents (S)-2-amino-2-methyldec-9-enoic acid or a stapled derivative
LSXETAXDLWKLLXEN

SEQ ID NO: 39 - protein, 16 aa, Artificial Sequence
  synthetic peptide synthesized by Fmoc-based solid phase peptide synthesis
  misc_feature (3)..(3): Xaa represents (S)-2-amino-2-methylhept-6-enoic acid or a stapled derivative
  misc_feature (7)..(7): Xaa represents 2-amino-2-(pent-4-enyl)hept-6-enoic acid or a stapled derivative
  misc_feature (14)..(14): Xaa represents (S)-2-amino-2-methyldec-9-enoic acid or a stapled derivative
LSXETFXDLWKLLXEN

SEQ ID NO: 40 - protein, 16 aa, Artificial Sequence
  synthetic peptide synthesized by Fmoc-based solid phase peptide synthesis
  misc_feature (3)..(3): Xaa represents (S)-2-amino-2-methylhept-6-enoic acid or a stapled derivative
  misc_feature (7)..(7): Xaa represents 2-amino-2-(pent-4-enyl)hept-6-enoic acid or a stapled derivative
  misc_feature (14)..(14): Xaa represents (S)-2-amino-2-methyldec-9-enoic acid or a stapled derivative
LSXETAXDLWKLLXEN

SEQ ID NO: 41 - protein, 16 aa, Artificial Sequence
  synthetic peptide synthesized by Fmoc-based solid phase peptide synthesis
  misc_feature (3)..(3): Xaa represents (S)-2-amino-2-methylhept-6-enoic acid or a stapled derivative
  misc_feature (7)..(7): Xaa represents 2-amino-2-(pent-4-enyl)hept-6-enoic acid or a stapled derivative
  misc_feature (14)..(14): Xaa represents (S)-2-amino-2-methyldec-9-enoic acid or a stapled derivative
LSXETFXDLWKLLXEN

SEQ ID NO: 42 - protein, 16 aa, Artificial Sequence
  synthetic peptide synthesized by Fmoc-based solid phase peptide synthesis
  misc_feature (3)..(3): Xaa represents (S)-2-amino-2-methylhept-6-enoic acid or a stapled derivative
  misc_feature (7)..(7): Xaa represents 2-amino-2-(pent-4-enyl)hept-6-enoic acid or a stapled derivative
  misc_feature (14)..(14): Xaa represents (S)-2-amino-2-methyldec-9-enoic acid or a stapled derivative
LSXETAXDLWKLLXEN

SEQ ID NO: 43 - protein, 10 aa, Artificial Sequence
  synthetic peptide synthesized by Fmoc-based solid phase peptide synthesis
  misc_feature (1)..(1): Xaa represents (S)-2-amino-2-methylhept-6-enoic acid or a stapled derivative
  misc_feature (5)..(5): Xaa represents 2-amino-2-(pent-4-enyl)hept-6-enoic acid or a stapled derivative
  misc_feature (9)..(9): Xaa represents (R)-2-amino-2-methylhept-6-enoic acid or a stapled derivative
XDFSXYWKXL

SEQ ID NO: 44 - protein, 10 aa, Artificial Sequence
  synthetic peptide synthesized by Fmoc-based solid phase peptide synthesis
  misc_feature (1)..(1): Xaa represents (R)-2-amino-2-methylhept-6-enoic acid or a stapled derivative
  misc_feature (5)..(5): Xaa represents 2-amino-2-(pent-4-enyl)hept-6-enoic acid or a stapled derivative
  misc_feature (9)..(9): Xaa represents (S)-2-amino-2-methylhept-6-enoic acid or a stapled derivative
XDFSXYWKXL

SEQ ID NO: 45 - protein, 22 aa, Artificial Sequence
  synthetic peptide synthesized by Fmoc-based solid phase peptide synthesis
  misc_feature (9)..(9): Xaa represents (S)-2-amino-2-methylhept-6-enoic acid or a stapled derivative
  misc_feature (13)..(13): Xaa represents 2-amino-2-(pent-4-enyl)hept-6-enoic acid or a stapled derivative
  misc_feature (18)..(18): Xaa represents Nle (Norleucine)
  misc_feature (20)..(20): Xaa represents (S)-2-amino-2-methyldec-9-enoic acid or a stapled derivative
EDIIRNIAXHLAXVGDWXDXSI

SEQ ID NO: 46 - protein, 17 aa, Artificial Sequence
  synthetic peptide synthesized by Fmoc-based solid phase peptide synthesis
  misc_feature (4)..(4): Xaa represents (S)-2-amino-2-methylhept-6-enoic acid or a stapled derivative
  misc_feature (8)..(8): Xaa represents 2-amino-2-(pent-4-enyl)hept-6-enoic acid or a stapled derivative
  misc_feature (13)..(13): Xaa represents Nle (Norleucine)
  misc_feature (15)..(15): Xaa represents (S)-2-amino-2-methyldec-9-enoic acid or a stapled derivative
NIAXHLAXVGDWXDXSI

SEQ ID NO: 47 - protein, 15 aa, Artificial Sequence
  synthetic peptide synthesized by Fmoc-based solid phase peptide synthesis
  misc_feature (4)..(4): Xaa represents (S)-2-amino-2-methylhept-6-enoic acid or a stapled derivative
  misc_feature (8)..(8): Xaa represents 2-amino-2-(pent-4-enyl)hept-6-enoic acid or a stapled derivative
  misc_feature (13)..(13): Xaa represents Nle (Norleucine)
  misc_feature (15)..(15): Xaa represents (S)-2-amino-2-methyldec-9-enoic acid or a stapled derivative
NIAXHLAXVGDWXDX

SEQ ID NO: 48 - protein, 22 aa, Artificial Sequence
  synthetic peptide synthesized by Fmoc-based solid phase peptide synthesis
  misc_feature (9)..(9): Xaa represents (S)-2-amino-2-methylhept-6-enoic acid or a stapled derivative
  misc_feature (13)..(13): Xaa represents 2-amino-2-(pent-4-enyl)hept-6-enoic acid or a stapled derivative
  misc_feature (18)..(18): Xaa represents Nle (Norleucine)
  misc_feature (20)..(20): Xaa represents (S)-2-amino-2-methyldec-9-enoic acid or a stapled derivative
EDIIRNIAXHLAXVGDWXDXSI

SEQ ID NO: 49 - protein, 17 aa, Artificial Sequence
  synthetic peptide synthesized by Fmoc-based solid phase peptide synthesis
  misc_feature (4)..(4): Xaa represents (S)-2-amino-2-methylhept-6-enoic acid or a stapled derivative
  misc_feature (8)..(8): Xaa represents 2-amino-2-(pent-4-enyl)hept-6-enoic acid or a stapled derivative
  misc_feature (13)..(13): Xaa represents Nle (Norleucine)
  misc_feature (15)..(15): Xaa represents (S)-2-amino-2-methyldec-9-enoic acid or a stapled derivative
NIAXHLAXVGDWXDXSI

SEQ ID NO: 50 - protein, 15 aa, Artificial Sequence
  synthetic peptide synthesized by Fmoc-based solid phase peptide synthesis
  misc_feature (4)..(4): Xaa represents (S)-2-amino-2-methylhept-6-enoic acid or a stapled derivative
  misc_feature (8)..(8): Xaa represents 2-amino-2-(pent-4-enyl)hept-6-enoic acid or a stapled derivative
  misc_feature (13)..(13): Xaa represents Nle (Norleucine)
  misc_feature (15)..(15): Xaa represents (S)-2-amino-2-methyldec-9-enoic acid or a stapled derivative
NIAXHLAXVGDWXDX

SEQ ID NO: 51 - protein, 21 aa, Artificial Sequence
  synthetic peptide synthesized by Fmoc-based solid phase peptide synthesis
  misc_feature (2)..(2): Xaa represents (S)-2-amino-2-methylhept-6-enoic acid or a stapled derivative
  misc_feature (6)..(6): Xaa represents 2-amino-2-(pent-4-enyl)hept-6-enoic acid or a stapled derivative
  misc_feature (10)..(10): Xaa represents (R)-2-amino-2-methylhept-6-enoic acid or a stapled derivative
LXILQXAVQXILGLEQQVRER

SEQ ID NO: 52 - protein, 21 aa, Artificial Sequence
  synthetic peptide synthesized by Fmoc-based solid phase peptide synthesis
  misc_feature (2)..(2): Xaa represents (S)-2-amino-2-methylhept-6-enoic acid or a stapled derivative
  misc_feature (6)..(6): Xaa represents 2-amino-2-(pent-4-enyl)hept-6-enoic acid or a stapled derivative
  misc_feature (13)..(13): Xaa represents (S)-2-amino-2-methyldec-9-enoic acid or a stapled derivative
LXILQXAVQVILXLEQQVRER

SEQ ID NO: 53 - protein, 21 aa, Artificial Sequence
  synthetic peptide synthesized by Fmoc-based solid phase peptide synthesis
  misc_feature (9)..(9): Xaa represents (S)-2-amino-2-methylhept-6-enoic acid or a stapled derivative
  misc_feature (13)..(13): Xaa represents 2-amino-2-(pent-4-enyl)hept-6-enoic acid or a stapled derivative
  misc_feature (17)..(17): Xaa represents (R)-2-amino-2-methylhept-6-enoic acid or a stapled derivative
LLILQQAVXVILXLEQXVRER

SEQ ID NO: 54 - protein, 21 aa, Artificial Sequence
  synthetic peptide synthesized by Fmoc-based solid phase peptide synthesis
  misc_feature (9)..(9): Xaa represents (S)-2-amino-2-methylhept-6-enoic acid or a stapled derivative
  misc_feature (13)..(13): Xaa represents 2-amino-2-(pent-4-enyl)hept-6-enoic acid or a stapled derivative
  misc_feature (20)..(20): Xaa represents (S)-2-amino-2-methyldec-9-enoic acid or a stapled derivative
LLILQQAVXVILXLEQQVRXR

SEQ ID NO: 55 - protein, 21 aa, Artificial Sequence
  synthetic peptide synthesized by Fmoc-based solid phase peptide synthesis
  misc_feature (5)..(5): Xaa represents (S)-2-amino-2-methylhept-6-enoic acid or a stapled derivative
  misc_feature (9)..(9): Xaa represents 2-amino-2-(pent-4-enyl)hept-6-enoic acid or a stapled derivative
  misc_feature (13)..(13): Xaa represents (R)-2-amino-2-methylhept-6-enoic acid or a stapled derivative
LLILXQAVXVILXLEQQVRER

SEQ ID NO: 56 - protein, 21 aa, Artificial Sequence
  synthetic peptide synthesized by Fmoc-based solid phase peptide synthesis
  misc_feature (5)..(5): Xaa represents (S)-2-amino-2-methylhept-6-enoic acid or a stapled derivative
  misc_feature (9)..(9): Xaa represents 2-amino-2-(pent-4-enyl)hept-6-enoic acid or a stapled derivative
  misc_feature (16)..(16): Xaa represents (S)-2-amino-2-methyldec-9-enoic acid or a stapled derivative
LLILXQAVXVILGLEXQVRER

SEQ ID NO: 57 - protein, 21 aa, Artificial Sequence
  synthetic peptide synthesized by Fmoc-based solid phase peptide synthesis
  misc_feature (5)..(5): Xaa represents (S)-2-amino-2-methylhept-6-enoic acid or a stapled derivative
  misc_feature (9)..(9): Xaa represents 2-amino-2-(pent-4-enyl)hept-6-enoic acid or a stapled derivative
  misc_feature (13)..(13): Xaa represents 2-amino-2-(pent-4-enyl)hept-6-enoic acid or a stapled derivative
  misc_feature (17)..(17): Xaa represents (S)-2-amino-2-methylhept-6-enoic acid or a stapled derivative
LLILXQAVXVILXLEQXVRER

SEQ ID NO: 58 - protein, 21 aa, Artificial Sequence
  synthetic peptide synthesized by Fmoc-based solid phase peptide synthesis
  misc_feature (2)..(2): Xaa represents (S)-2-amino-2-methylhept-6-enoic acid or a stapled derivative
  misc_feature (6)..(6): Xaa represents 2-amino-2-(pent-4-enyl)hept-6-enoic acid or a stapled derivative
  misc_feature (10)..(10): Xaa represents (R)-2-amino-2-methylhept-6-enoic acid or a stapled derivative
LXILQXAVQXILGLEQQVRER

SEQ ID NO: 59 - protein, 21 aa, Artificial Sequence
  synthetic peptide synthesized by Fmoc-based solid phase peptide synthesis
  misc_feature (2)..(2): Xaa represents (S)-2-amino-2-methylhept-6-enoic acid or a stapled derivative
  misc_feature (6)..(6): Xaa represents 2-amino-2-(pent-4-enyl)hept-6-enoic acid or a stapled derivative
  misc_feature (13)..(13): Xaa represents (S)-2-amino-2-methyldec-9-enoic acid or a stapled derivative
LXILQXAVQVILXLEQQVRER

SEQ ID NO: 60 - protein, 21 aa, Artificial Sequence
  synthetic peptide synthesized by Fmoc-based solid phase peptide synthesis
  misc_feature (9)..(9): Xaa represents (S)-2-amino-2-methylhept-6-enoic acid or a stapled derivative
  misc_feature (13)..(13): Xaa represents 2-amino-2-(pent-4-enyl)hept-6-enoic acid or a stapled derivative
  misc_feature (17)..(17): Xaa represents (R)-2-amino-2-methylhept-6-enoic acid or a stapled derivative
LLILQQAVXVILXLEQXVRER

SEQ ID NO: 61 - protein, 21 aa, Artificial Sequence
  synthetic peptide synthesized by Fmoc-based solid phase peptide synthesis
  misc_feature (9)..(9): Xaa represents (S)-2-amino-2-methylhept-6-enoic acid or a stapled derivative
  misc_feature (13)..(13): Xaa represents 2-amino-2-(pent-4-enyl)hept-6-enoic acid or a stapled derivative
  misc_feature (20)..(20): Xaa represents (S)-2-amino-2-methyldec-9-enoic acid or a stapled derivative
LLILQQAVXVILXLEQQVRXR

SEQ ID NO: 62 - protein, 21 aa, Artificial Sequence
  synthetic peptide synthesized by Fmoc-based solid phase peptide synthesis
  misc_feature (5)..(5): Xaa represents (S)-2-amino-2-methylhept-6-enoic acid or a stapled derivative
  misc_feature (9)..(9): Xaa represents 2-amino-2-(pent-4-enyl)hept-6-enoic acid or a stapled derivative
  misc_feature (13)..(13): Xaa represents (R)-2-amino-2-methylhept-6-enoic acid or a stapled derivative
LLILXQAVXVILXLEQQVRER

SEQ ID NO: 63 - protein, 21 aa, Artificial Sequence
  synthetic peptide synthesized by Fmoc-based solid phase peptide synthesis
  misc_feature (5)..(5): Xaa represents (S)-2-amino-2-methylhept-6-enoic acid or a stapled derivative
  misc_feature (9)..(9): Xaa represents 2-amino-2-(pent-4-enyl)hept-6-enoic acid or a stapled derivative
  misc_feature (16)..(16): Xaa represents (S)-2-amino-2-methyldec-9-enoic acid or a stapled derivative
LLILXQAVXVILGLEXQVRER

SEQ ID NO: 64 - protein, 21 aa, Artificial Sequence
  synthetic peptide synthesized by Fmoc-based solid phase peptide synthesis
  misc_feature (5)..(5): Xaa represents (S)-2-amino-2-methylhept-6-enoic acid or a stapled derivative
  misc_feature (9)..(9): Xaa represents 2-amino-2-(pent-4-enyl)hept-6-enoic acid or a stapled derivative
  misc_feature (13)..(13): Xaa represents 2-amino-2-(pent-4-enyl)hept-6-enoic acid or a stapled derivative
  misc_feature (17)..(17): Xaa represents (S)-2-amino-2-methylhept-6-enoic acid or a stapled derivative
LLILXQAVXVILXLEQXVRER

SEQ ID NO: 65 - protein, 30 aa, Artificial Sequence
  synthetic peptide synthesized by Fmoc-based solid phase peptide synthesis
  misc_feature (14)..(14): Xaa represents (S)-2-amino-2-methylhept-6-enoic acid or a stapled derivative
  misc_feature (18)..(18): Xaa represents 2-amino-2-(pent-4-enyl)hept-6-enoic acid or a stapled derivative
  misc_feature (22)..(22): Xaa represents 2-amino-2-(pent-4-enyl)hept-6-enoic acid or a stapled derivative
  misc_feature (26)..(26): Xaa represents (S)-2-amino-2-methylhept-6-enoic acid or a stapled derivative
HAEGTFTSDVSSYXEGQXAKEXIAWXVKGR

SEQ ID NO: 66 - protein, 30 aa, Artificial Sequence
  synthetic peptide synthesized by Fmoc-based solid phase peptide synthesis
  misc_feature (14)..(14): Xaa represents (S)-2-amino-2-methylhept-6-enoic acid or a stapled derivative
  misc_feature (18)..(18): Xaa represents 2-amino-2-(pent-4-enyl)hept-6-enoic acid or a stapled derivative
  misc_feature (25)..(25): Xaa represents (S)-2-amino-2-methyldec-9-enoic acid or a stapled derivative
HAEGTFTSDVSSYXEGQXAKEFIAXLVKGR

SEQ ID NO: 67 - protein, 30 aa, Artificial Sequence
  synthetic peptide synthesized by Fmoc-based solid phase peptide synthesis
  misc_feature (18)..(18): Xaa represents (S)-2-amino-2-methylhept-6-enoic acid or a stapled derivative
  misc_feature (22)..(22): Xaa represents 2-amino-2-(pent-4-enyl)hept-6-enoic acid or a stapled derivative
  misc_feature (29)..(29): Xaa represents (S)-2-amino-2-methyldec-9-enoic acid or a stapled derivative
HAEGTFTSDVSSYLEGQXAKEXIAWLVKXR

SEQ ID NO: 68 - protein, 30 aa, Artificial Sequence
  synthetic peptide synthesized by Fmoc-based solid phase peptide synthesis
  misc_feature (17)..(17): Xaa represents (S)-2-amino-2-methylhept-6-enoic acid or a stapled derivative
  misc_feature (21)..(21): Xaa represents 2-amino-2-(pent-4-enyl)hept-6-enoic acid or a stapled derivative
  misc_feature (25)..(25): Xaa represents 2-amino-2-(pent-4-enyl)hept-6-enoic acid or a stapled derivative
  misc_feature (29)..(29): Xaa represents (S)-2-amino-2-methylhept-6-enoic acid or a stapled derivative
HAEGTFTSDVSSYLEGXAAKXFIAXLVKXR

SEQ ID NO: 69 - protein, 30 aa, Artificial Sequence
  synthetic peptide synthesized by Fmoc-based solid phase peptide synthesis
  misc_feature (21)..(21): Xaa represents (S)-2-amino-2-methylhept-6-enoic acid or a stapled derivative
  misc_feature (25)..(25): Xaa represents 2-amino-2-(pent-4-enyl)hept-6-enoic acid or a stapled derivative
  misc_feature (29)..(29): Xaa represents (R)-2-amino-2-methylhept-6-enoic acid or a stapled derivative
HAEGTFTSDVSSYLEGQAAKXFIAXLVKXR

SEQ ID NO: 70 - protein, 30 aa, Artificial Sequence
  synthetic peptide synthesized by Fmoc-based solid phase peptide synthesis
  misc_feature (10)..(10): Xaa represents (R)-2-amino-2-methyldec-9-enoic acid or a stapled derivative
  misc_feature (17)..(17): Xaa represents 2-amino-2-(pent-4-enyl)hept-6-enoic acid or a stapled derivative
  misc_feature (24)..(24): Xaa represents (S)-2-amino-2-methyldec-9-enoic acid or a stapled derivative
HAEGTFTSDXSSYLEGXAAKEFIXWLVKGR

SEQ ID NO: 71 - protein, 30 aa, Artificial Sequence
  synthetic peptide synthesized by Fmoc-based solid phase peptide synthesis
  misc_feature (16)..(16): Xaa represents (S)-2-amino-2-methylhept-6-enoic acid or a stapled derivative
  misc_feature (20)..(20): Xaa represents 2-amino-2-(pent-4-enyl)hept-6-enoic acid or a stapled derivative
  misc_feature (27)..(27): Xaa represents (S)-2-amino-2-methyldec-9-enoic acid or a stapled derivative
HAEGTFTSDVSSYLEXQAAXEFIAWLXKGR

SEQ ID NO: 72 - protein, 30 aa, Artificial Sequence
  synthetic peptide synthesized by Fmoc-based solid phase peptide synthesis
  misc_feature (13)..(13): Xaa represents (R)-2-amino-2-methyldec-9-enoic acid or a stapled derivative
  misc_feature (20)..(20): Xaa represents 2-amino-2-(pent-4-enyl)hept-6-enoic acid or a stapled derivative
  misc_feature (27)..(27): Xaa represents (S)-2-amino-2-methyldec-9-enoic acid or a stapled derivative
HAEGTFTSDVSSXLEGQAAXEFIAWLXKGR

SEQ ID NO: 73 - protein, 30 aa, Artificial Sequence
  synthetic peptide synthesized by Fmoc-based solid phase peptide synthesis
  misc_feature (12)..(12): Xaa represents (S)-2-amino-2-methylhept-6-enoic acid or a stapled derivative
  misc_feature (16)..(16): Xaa represents 2-amino-2-(pent-4-enyl)hept-6-enoic acid or a stapled derivative
  misc_feature (23)..(23): Xaa represents (S)-2-amino-2-methyldec-9-enoic acid or a stapled derivative
HAEGTFTSDVSXYLEXQAAKEFXAWLVKGR

SEQ ID NO: 74 - protein, 30 aa, Artificial Sequence
  synthetic peptide synthesized by Fmoc-based solid phase peptide synthesis
  misc_feature (10)..(10): Xaa represents (S)-2-amino-2-methylhept-6-enoic acid or a stapled derivative
  misc_feature (14)..(14): Xaa represents 2-amino-2-(pent-4-enyl)hept-6-enoic acid or a stapled derivative
  misc_feature (21)..(21): Xaa represents (S)-2-amino-2-methyldec-9-enoic acid or a stapled derivative
HAEGTFTSDXSSYXEGQAAKXFIAWLVKGR

SEQ ID NO: 75 - protein, 30 aa, Artificial Sequence
  synthetic peptide synthesized by Fmoc-based solid phase peptide synthesis
  misc_feature (8)..(8): Xaa represents (S)-2-amino-2-methylhept-6-enoic acid or a stapled derivative
  misc_feature (12)..(12): Xaa represents 2-amino-2-(pent-4-enyl)hept-6-enoic acid or a stapled derivative
  misc_feature (19)..(19): Xaa represents (S)-2-amino-2-methyldec-9-enoic acid or a stapled derivative
HAEGTFTXDVSXYLEGQAXKEFIAWLVKGR

SEQ ID NO: 76 - protein, 30 aa, Artificial Sequence
  synthetic peptide synthesized by Fmoc-based solid phase peptide synthesis
  misc_feature (8)..(8): Xaa represents (S)-2-amino-2-methylhept-6-enoic acid or a stapled derivative
  misc_feature (12)..(12): Xaa represents 2-amino-2-(pent-4-enyl)hept-6-enoic acid or a stapled derivative
  misc_feature (16)..(16): Xaa represents (R)-2-amino-2-methylhept-6-enoic acid or a stapled derivative
HAEGTFTXDVSXYLEXQAAKEFIAWLVKGR

SEQ ID NO: 77 - protein, 30 aa, Artificial Sequence
  synthetic peptide synthesized by Fmoc-based solid phase peptide synthesis
  misc_feature (8)..(8): Xaa represents (S)-2-amino-2-methylhept-6-enoic acid or a stapled derivative
  misc_feature (12)..(12): Xaa represents 2-amino-2-(pent-4-enyl)hept-6-enoic acid or a stapled derivative
  misc_feature (16)..(16): Xaa represents 2-amino-2-(pent-4-enyl)hept-6-enoic acid or a stapled derivative
  misc_feature (20)..(20): Xaa represents (S)-2-amino-2-methylhept-6-enoic acid or a stapled derivative
HAEGTFTXDVSXYLEXQAAXEFIAWLVKGR

SEQ ID NO: 78 - protein, 30 aa, Artificial Sequence
  synthetic peptide synthesized by Fmoc-based solid phase peptide synthesis
  misc_feature (12)..(12): Xaa represents (S)-2-amino-2-methylhept-6-enoic acid or a stapled derivative
  misc_feature (16)..(16): Xaa represents 2-amino-2-(pent-4-enyl)hept-6-enoic acid or a stapled derivative
  misc_feature (20)..(20): Xaa represents (R)-2-amino-2-methylhept-6-enoic acid or a stapled derivative
HAEGTFTSDVSXYLEXQAAXEFIAWLVKGR

SEQ ID NO: 79 - protein, 27 aa, Artificial Sequence
  synthetic peptide synthesized by Fmoc-based solid phase peptide synthesis
  misc_feature (8)..(8): Xaa represents (S)-2-amino-2-methylhept-6-enoic acid or a stapled derivative
  misc_feature (12)..(12): Xaa represents 2-amino-2-(pent-4-enyl)hept-6-enoic acid or a stapled derivative
  misc_feature (19)..(19): Xaa represents (S)-2-amino-2-methyldec-9-enoic acid or a stapled derivative
SGSWLRDXWDWXCTVLTDXKTWLQSKL

SEQ ID NO: 80 - protein, 27 aa, Artificial Sequence
  synthetic peptide synthesized by Fmoc-based solid phase peptide synthesis
  misc_feature (13)..(13): Xaa represents (S)-2-amino-2-methylhept-6-enoic acid or a stapled derivative
  misc_feature (17)..(17): Xaa represents 2-amino-2-(pent-4-enyl)hept-6-enoic acid or a stapled derivative
  misc_feature (21)..(21): Xaa represents 2-amino-2-(pent-4-enyl)hept-6-enoic acid or a stapled derivative
  misc_feature (25)..(25): Xaa represents (S)-2-amino-2-methylhept-6-enoic acid or a stapled derivative
SGSWLRDVWDWIXTVLXDFKXWLQXKL

SEQ ID NO: 81 - protein, 27 aa, Artificial Sequence
  synthetic peptide synthesized by Fmoc-based solid phase peptide synthesis
  misc_feature (6)..(6): Xaa represents (S)-2-amino-2-methylhept-6-enoic acid or a stapled derivative
  misc_feature (10)..(10): Xaa represents 2-amino-2-(pent-4-enyl)hept-6-enoic acid or a stapled derivative
  misc_feature (17)..(17): Xaa represents (S)-2-amino-2-methyldec-9-enoic acid or a stapled derivative
SGSWLXDVWXWICTVLXDFKTWLQSKL

SEQ ID NO: 82 - protein, 27 aa, Artificial Sequence
  synthetic peptide synthesized by Fmoc-based solid phase peptide synthesis
  misc_feature (6)..(6): Xaa represents (S)-2-amino-2-methylhept-6-enoic acid or a stapled derivative
  misc_feature (10)..(10): Xaa represents 2-amino-2-(pent-4-enyl)hept-6-enoic acid or a stapled derivative
  misc_feature (14)..(14): Xaa represents (R)-2-amino-2-methylhept-6-enoic acid or a stapled derivative
SGSWLXDVWXWICXVLTDFKTWLQSKL

SEQ ID NO: 83 - protein, 27 aa, Artificial Sequence
  synthetic peptide synthesized by Fmoc-based solid phase peptide synthesis
  misc_feature (6)..(6): Xaa represents (S)-2-amino-2-methylhept-6-enoic acid or a stapled derivative
  misc_feature (10)..(10): Xaa represents 2-amino-2-(pent-4-enyl)hept-6-enoic acid or a stapled derivative
  misc_feature (14)..(14): Xaa represents 2-amino-2-(pent-4-enyl)hept-6-enoic acid or a stapled derivative
  misc_feature (18)..(18): Xaa represents (S)-2-amino-2-methylhept-6-enoic acid or a stapled derivative
SGSWLXDVWXWICXVLTXFKTWLQSKL

SEQ ID NO: 84 - protein, 27 aa, Artificial Sequence
  synthetic peptide synthesized by Fmoc-based solid phase peptide synthesis
  misc_feature (10)..(10): Xaa represents (S)-2-amino-2-methylhept-6-enoic acid or a stapled derivative
  misc_feature (14)..(14): Xaa represents 2-amino-2-(pent-4-enyl)hept-6-enoic acid or a stapled derivative
  misc_feature (21)..(21): Xaa represents (S)-2-amino-2-methyldec-9-enoic acid or a stapled derivative
SGSWLRDVWXWICXVLTDFKXWLQSKL

SEQ ID NO: 85 - protein, 27 aa, Artificial Sequence
  synthetic peptide synthesized by Fmoc-based solid phase peptide synthesis
  misc_feature (10)..(10): Xaa represents (S)-2-amino-2-methylhept-6-enoic acid or a stapled derivative
  misc_feature (14)..(14): Xaa represents 2-amino-2-(pent-4-enyl)hept-6-enoic acid or a stapled derivative
  misc_feature (18)..(18): Xaa represents (R)-2-amino-2-methylhept-6-enoic acid or a stapled derivative
SGSWLRDVWXWICXVLTXFKTWLQSKL

SEQ ID NO: 86 - protein, 27 aa, Artificial Sequence
  synthetic peptide synthesized by Fmoc-based solid phase peptide synthesis
  misc_feature (7)..(7): Xaa represents (R)-2-amino-2-methyldec-9-enoic acid or a stapled derivative
  misc_feature (14)..(14): Xaa represents 2-amino-2-(pent-4-enyl)hept-6-enoic acid or a stapled derivative
  misc_feature (21)..(21): Xaa represents (S)-2-amino-2-methyldec-9-enoic acid or a stapled derivative
SGSWLRXVWDWICXVLTDFKXWLQSKL

SEQ ID NO: 87 - protein, 27 aa, Artificial Sequence
  synthetic peptide synthesized by Fmoc-based solid phase peptide synthesis
  misc_feature (8)..(8): Xaa represents (S)-2-amino-2-methylhept-6-enoic acid or a stapled derivative
  misc_feature (12)..(12): Xaa represents 2-amino-2-(pent-4-enyl)hept-6-enoic acid or a stapled derivative
  misc_feature (19)..(19): Xaa represents (S)-2-amino-2-methyldec-9-enoic acid or a stapled derivative
SGSWLRDXWDWXCTVLTDXKTWLQSKL

SEQ ID NO: 88 - protein, 27 aa, Artificial Sequence
  synthetic peptide synthesized by Fmoc-based solid phase peptide synthesis
  misc_feature (13)..(13): Xaa represents (S)-2-amino-2-methylhept-6-enoic acid or a stapled derivative
  misc_feature (17)..(17): Xaa represents 2-amino-2-(pent-4-enyl)hept-6-enoic acid or a stapled derivative
  misc_feature (21)..(21): Xaa represents 2-amino-2-(pent-4-enyl)hept-6-enoic acid or a stapled derivative
  misc_feature (25)..(25): Xaa represents (S)-2-amino-2-methylhept-6-enoic acid or a stapled derivative
SGSWLRDVWDWIXTVLXDFKXWLQXKL

SEQ ID NO: 89 - protein, 27 aa, Artificial Sequence
  synthetic peptide synthesized by Fmoc-based solid phase peptide synthesis
  misc_feature (6)..(6): Xaa represents (S)-2-amino-2-methylhept-6-enoic acid or a stapled derivative
  misc_feature (10)..(10): Xaa represents 2-amino-2-(pent-4-enyl)hept-6-enoic acid or a stapled derivative
  misc_feature (17)..(17): Xaa represents (S)-2-amino-2-methyldec-9-enoic acid or a stapled derivative
SGSWLXDVWXWICTVLXDFKTWLQSKL

SEQ ID NO: 90 - protein, 27 aa, Artificial Sequence
  synthetic peptide synthesized by Fmoc-based solid phase peptide synthesis
  misc_feature (6)..(6): Xaa represents (S)-2-amino-2-methylhept-6-enoic acid or a stapled derivative
  misc_feature (10)..(10): Xaa represents 2-amino-2-(pent-4-enyl)hept-6-enoic acid or a stapled derivative
  misc_feature (14)..(14): Xaa represents (R)-2-amino-2-methylhept-6-enoic acid or a stapled derivative
SGSWLXDVWXWICXVLTDFKTWLQSKL

SEQ ID NO: 91 - protein, 27 aa, Artificial Sequence
  synthetic peptide synthesized by Fmoc-based solid phase peptide synthesis
  misc_feature (6)..(6): Xaa represents (S)-2-amino-2-methylhept-6-enoic acid or a stapled derivative
  misc_feature (10)..(10): Xaa represents 2-amino-2-(pent-4-enyl)hept-6-enoic acid or a stapled derivative
  misc_feature (14)..(14): Xaa represents 2-amino-2-(pent-4-enyl)hept-6-enoic acid or a stapled derivative
  misc_feature (18)..(18): Xaa represents (S)-2-amino-2-methylhept-6-enoic acid or a stapled derivative
SGSWLXDVWXWICXVLTXFKTWLQSKL

SEQ ID NO: 92 - protein, 27 aa, Artificial Sequence
  synthetic peptide synthesized by Fmoc-based solid phase peptide synthesis
  misc_feature (10)..(10): Xaa represents (S)-2-amino-2-methylhept-6-enoic acid or a stapled derivative
  misc_feature (14)..(14): Xaa represents 2-amino-2-(pent-4-enyl)hept-6-enoic acid or a stapled derivative
  misc_feature (21)..(21): Xaa represents (S)-2-amino-2-methyldec-9-enoic acid or a stapled derivative
SGSWLRDVWXWICXVLTDFKXWLQSKL

SEQ ID NO: 93 - protein, 27 aa, Artificial Sequence
  synthetic peptide synthesized by Fmoc-based solid phase peptide synthesis
  misc_feature (10)..(10): Xaa represents (S)-2-amino-2-methylhept-6-enoic acid or a stapled derivative
  misc_feature (14)..(14): Xaa represents 2-amino-2-(pent-4-enyl)hept-6-enoic acid or a stapled derivative
  misc_feature (18)..(18): Xaa represents (R)-2-amino-2-methylhept-6-enoic acid or a stapled derivative
SGSWLRDVWXWICXVLTXFKTWLQSKL

SEQ ID NO: 94 - protein, 27 aa, Artificial Sequence
  synthetic peptide synthesized by Fmoc-based solid phase peptide synthesis
  misc_feature (7)..(7): Xaa represents (R)-2-amino-2-methyldec-9-enoic acid or a stapled derivative
  misc_feature (14)..(14): Xaa represents 2-amino-2-(pent-4-enyl)hept-6-enoic acid or a stapled derivative
  misc_feature (21)..(21): Xaa represents (S)-2-amino-2-methyldec-9-enoic acid or a stapled derivative
SGSWLRXVWDWICXVLTDFKXWLQSKL

SEQ ID NO: 95 - protein, 27 aa, Artificial Sequence
  synthetic peptide synthesized by Fmoc-based solid phase peptide synthesis -linker1
  misc_feature (8)..(8): Xaa represents (S)-2-amino-2-methylhept-6-enoic acid or a stapled derivative
  misc_feature (12)..(12): Xaa represents 2-amino-2-(pent-4-enyl)hept-6-enoic acid or a stapled derivative
  misc_feature (19)..(19): Xaa represents (S)-2-amino-2-methyldec-9-enoic acid or a stapled derivative
SGSWLRDXWDWXCTVLTDXKTWLQSKL

SEQ ID NO: 96 - protein, 27 aa, Artificial Sequence
  synthetic peptide synthesized by Fmoc-based solid phase peptide synthesis -linker1
  misc_feature (13)..(13): Xaa represents (S)-2-amino-2-methylhept-6-enoic acid or a stapled derivative
  misc_feature (17)..(17): Xaa represents 2-amino-2-(pent-4-enyl)hept-6-enoic acid or a stapled derivative
  misc_feature (21)..(21): Xaa represents 2-amino-2-(pent-4-enyl)hept-6-enoic acid or a stapled derivative
  misc_feature (25)..(25): Xaa represents (S)-2-amino-2-methylhept-6-enoic acid or a stapled derivative
SGSWLRDVWDWIXTVLXDFKXWLQXKL

SEQ ID NO: 97 - protein, 27 aa, Artificial Sequence
  synthetic peptide synthesized by Fmoc-based solid phase peptide synthesis -linker1
  misc_feature (6)..(6): Xaa represents (S)-2-amino-2-methylhept-6-enoic acid or a stapled derivative
  misc_feature (10)..(10): Xaa represents 2-amino-2-(pent-4-enyl)hept-6-enoic acid or a stapled derivative
  misc_feature (17)..(17): Xaa represents (S)-2-amino-2-methyldec-9-enoic acid or a stapled derivative
SGSWLXDVWXWICTVLXDFKTWLQSKL

SEQ ID NO: 98 - protein, 27 aa, Artificial Sequence
  synthetic peptide synthesized by Fmoc-based solid phase peptide synthesis -linker1
  misc_feature (6)..(6): Xaa represents (S)-2-amino-2-methylhept-6-enoic acid or a stapled derivative
  misc_feature (10)..(10): Xaa represents 2-amino-2-(pent-4-enyl)hept-6-enoic acid or a stapled derivative
  misc_feature (14)..(14): Xaa represents (R)-2-amino-2-methylhept-6-enoic acid or a stapled derivative
SGSWLXDVWXWICXVLTDFKTWLQSKL

SEQ ID NO: 99 - protein, 27 aa, Artificial Sequence
  synthetic peptide synthesized by Fmoc-based solid phase peptide synthesis -linker1
  misc_feature (6)..(6): Xaa represents (S)-2-amino-2-methylhept-6-enoic acid or a stapled derivative
  misc_feature (10)..(10): Xaa represents 2-amino-2-(pent-4-enyl)hept-6-enoic acid or a stapled derivative
  misc_feature (14)..(14): Xaa represents 2-amino-2-(pent-4-enyl)hept-6-enoic acid or a stapled derivative
  misc_feature (18)..(18): Xaa represents (S)-2-amino-2-methylhept-6-enoic acid or a stapled derivative
SGSWLXDVWXWICXVLTXFKTWLQSKL

SEQ ID NO: 100 - protein, 27 aa, Artificial Sequence
  synthetic peptide synthesized by Fmoc-based solid phase peptide synthesis -linker1
  misc_feature (10)..(10): Xaa represents (S)-2-amino-2-methylhept-6-enoic acid or a stapled derivative
  misc_feature (14)..(14): Xaa represents 2-amino-2-(pent-4-enyl)hept-6-enoic acid or a stapled derivative
  misc_feature (21)..(21): Xaa represents (S)-2-amino-2-methyldec-9-enoic acid or a stapled derivative
SGSWLRDVWXWICXVLTDFKXWLQSKL

SEQ ID NO: 101 - protein, 27 aa, Artificial Sequence
  synthetic peptide synthesized by Fmoc-based solid phase peptide synthesis -linker1
  misc_feature (10)..(10): Xaa represents (S)-2-amino-2-methylhept-6-enoic acid or a stapled derivative
  misc_feature (14)..(14): Xaa represents 2-amino-2-(pent-4-enyl)hept-6-enoic acid or a stapled derivative
  misc_feature (18)..(18): Xaa represents (R)-2-amino-2-methylhept-6-enoic acid or a stapled derivative
SGSWLRDVWXWICXVLTXFKTWLQSKL

SEQ ID NO: 102 - protein, 27 aa, Artificial Sequence
  synthetic peptide synthesized by Fmoc-based solid phase peptide synthesis -linker1
  misc_feature (7)..(7): Xaa represents (R)-2-amino-2-methyldec-9-enoic acid or a stapled derivative
  misc_feature (14)..(14): Xaa represents 2-amino-2-(pent-4-enyl)hept-6-enoic acid or a stapled derivative
  misc_feature (21)..(21): Xaa represents (S)-2-amino-2-methyldec-9-enoic acid or a stapled derivative
SGSWLRXVWDWICXVLTDFKXWLQSKL

SEQ ID NO: 103 - protein, 27 aa, Artificial Sequence
  synthetic peptide synthesized by Fmoc-based solid phase peptide synthesis
  misc_feature (8)..(8): Xaa represents (S)-2-amino-2-methylhept-6-enoic acid or a stapled derivative
  misc_feature (12)..(12): Xaa represents 2-amino-2-(pent-4-enyl)hept-6-enoic acid or a stapled derivative
  misc_feature (19)..(19): Xaa represents (S)-2-amino-2-methyldec-9-enoic acid or a stapled derivative
SGSWLRDXWDWXCTVLTDXKTWLQSKL

SEQ ID NO: 104 - protein, 27 aa, Artificial Sequence
  synthetic peptide synthesized by Fmoc-based solid phase peptide synthesis
  misc_feature (13)..(13): Xaa represents (S)-2-amino-2-methylhept-6-enoic acid or a stapled derivative
  misc_feature (17)..(17): Xaa represents 2-amino-2-(pent-4-enyl)hept-6-enoic acid or a stapled derivative
  misc_feature (21)..(21): Xaa represents 2-amino-2-(pent-4-enyl)hept-6-enoic acid or a stapled derivative
  misc_feature (25)..(25): Xaa represents (S)-2-amino-2-methylhept-6-enoic acid or a stapled derivative
SGSWLRDVWDWIXTVLXDFKXWLQXKL

SEQ ID NO: 105 - protein, 27 aa, Artificial Sequence
  synthetic peptide synthesized by Fmoc-based solid phase peptide synthesis
  misc_feature (6)..(6): Xaa represents (S)-2-amino-2-methylhept-6-enoic acid or a stapled derivative
  misc_feature (10)..(10): Xaa represents 2-amino-2-(pent-4-enyl)hept-6-enoic acid or a stapled derivative
  misc_feature (17)..(17): Xaa represents (S)-2-amino-2-methyldec-9-enoic acid or a stapled derivative
SGSWLXDVWXWICTVLXDFKTWLQSKL

SEQ ID NO: 106 - protein, 27 aa, Artificial Sequence
  synthetic peptide synthesized by Fmoc-based solid phase peptide synthesis
  misc_feature (6)..(6): Xaa represents (S)-2-amino-2-methylhept-6-enoic acid or a stapled derivative
  misc_feature (10)..(10): Xaa represents 2-amino-2-(pent-4-enyl)hept-6-enoic acid or a stapled derivative
  misc_feature (14)..(14): Xaa represents (R)-2-amino-2-methylhept-6-enoic acid or a stapled derivative
SGSWLXDVWXWICXVLTDFKTWLQSKL

SEQ ID NO: 107 - protein, 27 aa, Artificial Sequence
  synthetic peptide synthesized by Fmoc-based solid phase peptide synthesis
  misc_feature (6)..(6): Xaa represents (S)-2-amino-2-methylhept-6-enoic acid or a stapled derivative
  misc_feature (10)..(10): Xaa represents 2-amino-2-(pent-4-enyl)hept-6-enoic acid or a stapled derivative
  misc_feature (14)..(14): Xaa represents 2-amino-2-(pent-4-enyl)hept-6-enoic acid or a stapled derivative
  misc_feature (18)..(18): Xaa represents (S)-2-amino-2-methylhept-6-enoic acid or a stapled derivative
SGSWLXDVWXWICXVLTXFKTWLQSKL

SEQ ID NO: 108 - protein, 27 aa, Artificial Sequence
  synthetic peptide synthesized by Fmoc-based solid phase peptide synthesis
  misc_feature (10)..(10): Xaa represents (S)-2-amino-2-methylhept-6-enoic acid or a stapled derivative
  misc_feature (14)..(14): Xaa represents 2-amino-2-(pent-4-enyl)hept-6-enoic acid or a stapled derivative
  misc_feature (21)..(21): Xaa represents (S)-2-amino-2-methyldec-9-enoic acid or a stapled derivative
SGSWLRDVWXWICXVLTDFKXWLQSKL

SEQ ID NO: 109 - protein, 27 aa, Artificial Sequence
  synthetic peptide synthesized by Fmoc-based solid phase peptide synthesis
  misc_feature (10)..(10): Xaa represents (S)-2-amino-2-methylhept-6-enoic acid or a stapled derivative
  misc_feature (14)..(14): Xaa represents 2-amino-2-(pent-4-enyl)hept-6-enoic acid or a stapled derivative
  misc_feature (18)..(18): Xaa represents (R)-2-amino-2-methylhept-6-enoic acid or a stapled derivative
SGSWLRDVWXWICXVLTXFKTWLQSKL

SEQ ID NO: 110 - protein, 27 aa, Artificial Sequence
  synthetic peptide synthesized by Fmoc-based solid phase peptide synthesis
  misc_feature (7)..(7): Xaa represents (R)-2-amino-2-methylhept-6-enoic acid or a stapled derivative
  misc_feature (14)..(14): Xaa represents 2-amino-2-(pent-4-enyl)hept-6-enoic acid or a stapled derivative
  misc_feature (21)..(21): Xaa represents (S)-2-amino-2-methyldec-9-enoic acid or a stapled derivative
SGSWLRXVWDWICXVLTDFKXWLQSKL

SEQ ID NO: 111 - protein, 27 aa, Artificial Sequence
  synthetic peptide synthesized by Fmoc-based solid phase peptide synthesis
  misc_feature (8)..(8): Xaa represents (S)-2-amino-2-methylhept-6-enoic acid or a stapled derivative
  misc_feature (12)..(12): Xaa represents 2-amino-2-(pent-4-enyl)hept-6-enoic acid or a stapled derivative
  misc_feature (19)..(19): Xaa represents (S)-2-amino-2-methyldec-9-enoic acid or a stapled derivative
SGSWLRDXWDWXCTVLTDXKTWLQSKL

SEQ ID NO: 112 - protein, 27 aa, Artificial Sequence
  synthetic peptide synthesized by Fmoc-based solid phase peptide synthesis
  misc_feature (13)..(13): Xaa represents (S)-2-amino-2-methylhept-6-enoic acid or a stapled derivative
  misc_feature (17)..(17): Xaa represents 2-amino-2-(pent-4-enyl)hept-6-enoic acid or a stapled derivative
  misc_feature (21)..(21): Xaa represents 2-amino-2-(pent-4-enyl)hept-6-enoic acid or a stapled derivative
  misc_feature (25)..(25): Xaa represents (S)-2-amino-2-methylhept-6-enoic acid or a stapled derivative
SGSWLRDVWDWIXTVLXDFKXWLQXKL

SEQ ID NO: 113 - protein, 27 aa, Artificial Sequence
  synthetic peptide synthesized by Fmoc-based solid phase peptide synthesis
  misc_feature (6)..(6): Xaa represents (S)-2-amino-2-methylhept-6-enoic acid or a stapled derivative
  misc_feature (10)..(10): Xaa represents 2-amino-2-(pent-4-enyl)hept-6-enoic acid or a stapled derivative
  misc_feature (17)..(17): Xaa represents (S)-2-amino-2-methyldec-9-enoic acid or a stapled derivative
SGSWLXDVWXWICTVLXDFKTWLQSKL

SEQ ID NO: 114 - protein, 27 aa, Artificial Sequence
  synthetic peptide synthesized by Fmoc-based solid phase peptide synthesis
  misc_feature (6)..(6): Xaa represents (S)-2-amino-2-methylhept-6-enoic acid or a stapled derivative
  misc_feature (10)..(10): Xaa represents 2-amino-2-(pent-4-enyl)hept-6-enoic acid or a stapled derivative
  misc_feature (14)..(14): Xaa represents (R)-2-amino-2-methylhept-6-enoic acid or a stapled derivative
SGSWLXDVWXWICXVLTDFKTWLQSKL

SEQ ID NO: 115 - protein, 27 aa, Artificial Sequence
  synthetic peptide synthesized by Fmoc-based solid phase peptide synthesis
  misc_feature (6)..(6): Xaa represents (S)-2-amino-2-methylhept-6-enoic acid or a stapled derivative
  misc_feature (10)..(10): Xaa represents 2-amino-2-(pent-4-enyl)hept-6-enoic acid or a stapled derivative
  misc_feature (14)..(14): Xaa represents 2-amino-2-(pent-4-enyl)hept-6-enoic acid or a stapled derivative
  misc_feature (18)..(18): Xaa represents (S)-2-amino-2-methylhept-6-enoic acid or a stapled derivative
SGSWLXDVWXWICXVLTXFKTWLQSKL

SEQ ID NO: 116 - protein, 27 aa, Artificial Sequence
  synthetic peptide synthesized by Fmoc-based solid phase peptide synthesis
  misc_feature (10)..(10): Xaa represents (S)-2-amino-2-methylhept-6-enoic acid or a stapled derivative
  misc_feature (14)..(14): Xaa represents 2-amino-2-(pent-4-enyl)hept-6-enoic acid or a stapled derivative
  misc_feature (21)..(21): Xaa represents (S)-2-amino-2-methyldec-9-enoic acid or a stapled derivative
SGSWLRDVWXWICXVLTDFKXWLQSKL

SEQ ID NO: 117 - protein, 27 aa, Artificial Sequence
  synthetic peptide synthesized by Fmoc-based solid phase peptide synthesis
  misc_feature (10)..(10): Xaa represents (S)-2-amino-2-methylhept-6-enoic acid or a stapled derivative
  misc_feature (14)..(14): Xaa represents 2-amino-2-(pent-4-enyl)hept-6-enoic acid or a stapled derivative
  misc_feature (18)..(18): Xaa represents (R)-2-amino-2-methylhept-6-enoic acid or a stapled derivative
SGSWLRDVWXWICXVLTXFKTWLQSKL

SEQ ID NO: 118 - protein, 27 aa, Artificial Sequence
  synthetic peptide synthesized by Fmoc-based solid phase peptide synthesis
  misc_feature (7)..(7): Xaa represents (R)-2-amino-2-methyldec-9-enoic acid or a stapled derivative
  misc_feature (14)..(14): Xaa represents 2-amino-2-(pent-4-enyl)hept-6-enoic acid or a stapled derivative
  misc_feature (21)..(21): Xaa represents (S)-2-amino-2-methyldec-9-enoic acid or a stapled derivative
SGSWLRXVWDWICXVLTDFKXWLQSKL

SEQ ID NO: 119 - protein, 24 aa, Artificial Sequence
  synthetic peptide synthesized by Fmoc-based solid phase peptide synthesis
  misc_feature (11)..(11): Xaa represents (S)-2-amino-2-methylhept-6-enoic acid or a stapled derivative
  misc_feature (15)..(15): Xaa represents 2-amino-2-(pent-4-enyl)hept-6-enoic acid or a stapled derivative
  misc_feature (22)..(22): Xaa represents (S)-2-amino-2-methyldec-9-enoic acid or a stapled derivative
KATEYIQYNLXRKNXTHQQDIXDL

SEQ ID NO: 120 - protein, 24 aa, Artificial Sequence
  synthetic peptide synthesized by Fmoc-based solid phase peptide synthesis
  misc_feature (7)..(7): Xaa represents (R)-2-amino-2-methyldec-9-enoic acid or a stapled derivative
  misc_feature (15)..(15): Xaa represents 2-amino-2-(pent-4-enyl)hept-6-enoic acid or a stapled derivative
  misc_feature (22)..(22): Xaa represents (S)-2-amino-2-methyldec-9-enoic acid or a stapled derivative
KATEYIXYNLRRKNXTHQQDIXDL

SEQ ID NO: 121 - protein, 23 aa, Artificial Sequence
  synthetic peptide synthesized by Fmoc-based solid phase peptide synthesis
  misc_feature (10)..(10): Xaa represents (S)-2-amino-2-methylhept-6-enoic acid or a stapled derivative
  misc_feature (14)..(14): Xaa represents 2-amino-2-(pent-4-enyl)hept-6-enoic acid or a stapled derivative
  misc_feature (21)..(21): Xaa represents (S)-2-amino-2-methyldec-9-enoic acid or a stapled derivative
TILKASVDYXRKLXREQQRAXEL

SEQ ID NO: 122 - protein, 23 aa, Artificial Sequence
  synthetic peptide synthesized by Fmoc-based solid phase peptide synthesis
  misc_feature (7)..(7): Xaa represents (R)-2-amino-2-methyldec-9-enoic acid or a stapled derivative
  misc_feature (14)..(14): Xaa represents 2-amino-2-(pent-4-enyl)hept-6-enoic acid or a stapled derivative
  misc_feature (21)..(21): Xaa represents (S)-2-amino-2-methyldec-9-enoic acid or a stapled derivative
TILKASXDYIRKLXREQQRAXEL

SEQ ID NO: 123 - protein, 13 aa, Artificial Sequence
  synthetic peptide synthesized by Fmoc-based solid phase peptide synthesis
  misc_feature (1)..(1): Xaa represents (S)-2-amino-2-methylhept-6-enoic acid or a stapled derivative
  misc_feature (5)..(5): Xaa represents 2-amino-2-(pent-4-enyl)hept-6-enoic acid or a stapled derivative
  misc_feature (9)..(9): Xaa represents 2-amino-2-(pent-4-enyl)hept-6-enoic acid or a stapled derivative
  misc_feature (13)..(13): Xaa represents (S)-2-amino-2-methylhept-6-enoic acid or a stapled derivative
XAAAXAAAXAAAX

SEQ ID NO: 124 - protein, 23 aa, Artificial Sequence
  synthetic peptide synthesized by Fmoc-based solid phase peptide synthesis
  misc_feature (13)..(13): Xaa represents (S)-2-amino-2-methylhept-6-enoic acid or a stapled derivative
  misc_feature (18)..(18): Xaa represents Nle (Norleucine)
EDIIRNIARHLAXVGDSXDRSIW

SEQ ID NO: 125 - protein, 18 aa, Artificial Sequence
  synthetic peptide synthesized by Fmoc-based solid phase peptide synthesis
  misc_feature (8)..(8): Xaa represents (S)-2-amino-2-methylhept-6-enoic acid or a stapled derivative
  misc_feature (13)..(13): Xaa represents Nle (Norleucine)
NIARHLAXVGDSXDRSIW

SEQ ID NO: 126 - protein, 22 aa, Artificial Sequence
  synthetic peptide synthesized by Fmoc-based solid phase peptide synthesis
  misc_feature (9)..(9): Xaa represents (S)-2-amino-2-methylhept-6-enoic acid or a stapled derivative
  misc_feature (13)..(13): Xaa represents 2-amino-2-(pent-4-enyl)hept-6-enoic acid or a stapled derivative
  misc_feature (18)..(18): Xaa represents Nle (Norleucine)
  misc_feature (20)..(20): Xaa represents (S)-2-amino-2-methyldec-9-enoic acid or a stapled derivative
EDIIRNIAXHLAXVGDSXDXSI

SEQ ID NO: 127 - protein, 17 aa, Artificial Sequence
  synthetic peptide synthesized by Fmoc-based solid phase peptide synthesis
  misc_feature (4)..(4): Xaa represents (S)-2-amino-2-methylhept-6-enoic acid or a stapled derivative
  misc_feature (8)..(8): Xaa represents 2-amino-2-(pent-4-enyl)hept-6-enoic acid or a stapled derivative
  misc_feature (13)..(13): Xaa represents Nle (Norleucine)
  misc_feature (15)..(15): Xaa represents (S)-2-amino-2-methyldec-9-enoic acid or a stapled derivative
NIAXHLAXVGDSXDXSI

SEQ ID NO: 128 - protein, 15 aa, Artificial Sequence
  synthetic peptide synthesized by Fmoc-based solid phase peptide synthesis
  misc_feature (4)..(4): Xaa represents (S)-2-amino-2-methylhept-6-enoic acid or a stapled derivative
  misc_feature (8)..(8): Xaa represents 2-amino-2-(pent-4-enyl)hept-6-enoic acid or a stapled derivative
  misc_feature (13)..(13): Xaa represents Nle (Norleucine)
  misc_feature (15)..(15): Xaa represents (S)-2-amino-2-methyldec-9-enoic acid or a stapled derivative
NIAXHLAXVGDSXDX